European Patent Application EP 4 219 555 A1, published August 2, 2023. Title: ANTIBODIES AND METHODS OF USE. Applicant: F. Hoffmann-La Roche AG. The sequence listing filed with the application follows.

SEQUENCE LISTING (166 sequences)

SEQ ID NO: 1 - protein, 5 aa, synthetic construct
  REGION 1..5: note = source = /note="Description of Artificial Sequence: Syntheticpeptide"
SYGIS

SEQ ID NO: 2 - protein, 5 aa, synthetic construct
  REGION 1..5: note = source = /note="Description of Artificial Sequence: Syntheticpeptide"
DYYMN

SEQ ID NO: 3 - protein, 5 aa, synthetic construct
  REGION 1..5: note = source = /note="Description of Artificial Sequence: Syntheticpeptide"
NYGVS

SEQ ID NO: 4 - protein, 5 aa, synthetic construct
  REGION 1..5: note = source = /note="Description of Artificial Sequence: Syntheticpeptide"
DTYMN

SEQ ID NO: 5 - protein, 5 aa, synthetic construct
  REGION 1..5: note = source = /note="Description of Artificial Sequence: Syntheticpeptide"
DTYIH

SEQ ID NO: 6 - protein, 5 aa, synthetic construct
  REGION 1..5: note = source = /note="Description of Artificial Sequence: Syntheticpeptide"
SYWIH

SEQ ID NO: 7 - protein, 5 aa, synthetic construct
  REGION 1..5: note = source = /note="Description of Artificial Sequence: Syntheticpeptide"
DTFTH

SEQ ID NO: 8 - protein, 5 aa, synthetic construct
  REGION 1..5: note = source = /note="Description of Artificial Sequence: Syntheticpeptide"
EYTMN

SEQ ID NO: 9 - protein, 5 aa, synthetic construct
  REGION 1..5: note = source = /note="Description of Artificial Sequence: Syntheticpeptide"
SYWIE

SEQ ID NO: 10 - protein, 5 aa, synthetic construct
  REGION 1..5: note = source = /note="Description of Artificial Sequence: Syntheticpeptide"
DYEMH

SEQ ID NO: 11 - protein, 5 aa, synthetic construct
  REGION 1..5: note = source = /note="Description of Artificial Sequence: Syntheticpeptide"
DTYIH

SEQ ID NO: 12 - protein, 5 aa, synthetic construct
  REGION 1..5: note = source = /note="Description of Artificial Sequence: Syntheticpeptide"
RYWMS

SEQ ID NO: 13 - protein, 5 aa, synthetic construct
  REGION 1..5: note = source = /note="Description of Artificial Sequence: Syntheticpeptide"
NYGMN

SEQ ID NO: 14 - protein, 7 aa, synthetic construct
  REGION 1..7: note = source = /note="Description of Artificial Sequence: Syntheticpeptide"
TSAMGIG

SEQ ID NO: 15 - protein, 5 aa, synthetic construct
  REGION 1..5: note = source = /note="Description of Artificial Sequence: Syntheticpeptide"
TYGVH

SEQ ID NO: 16 - protein, 17 aa, synthetic construct
  REGION 1..17: note = source = /note="Description of Artificial Sequence: Syntheticpeptide"
TVSSGGRYTYYPDSVKG

SEQ ID NO: 17 - protein, 17 aa, synthetic construct
  REGION 1..17: note = source = /note="Description of Artificial Sequence: Syntheticpeptide"
WIDPENDDTIYDPKFQG

SEQ ID NO: 18 - protein, 16 aa, synthetic construct
  REGION 1..16: note = source = /note="Description of Artificial Sequence: Syntheticpeptide"
VIWGDGSINYHSALIS

SEQ ID NO: 19 - protein, 17 aa, synthetic construct
  REGION 1..17: note = source = /note="Description of Artificial Sequence: Syntheticpeptide"
RIDPSNGNAKYDPKFQG

SEQ ID NO: 20 - protein, 17 aa, synthetic construct
  REGION 1..17: note = source = /note="Description of Artificial Sequence: Syntheticpeptide"
RIDPANGNTKYDPKFQD

SEQ ID NO: 21 - protein, 17 aa, synthetic construct
  REGION 1..17: note = source = /note="Description of Artificial Sequence: Syntheticpeptide"
EIDPSVSNSNYNQKFKG

SEQ ID NO: 22 - protein, 17 aa, synthetic construct
  REGION 1..17: note = source = /note="Description of Artificial Sequence: Syntheticpeptide"
RIDPSNGNTKYDPKFQG

SEQ ID NO: 23 - protein, 17 aa, synthetic construct
  REGION 1..17: note = source = /note="Description of Artificial Sequence: Syntheticpeptide"
GINPNNGETSYNQKFKG

SEQ ID NO: 24 - protein, 17 aa, synthetic construct
  REGION 1..17: note = source = /note="Description of Artificial Sequence: Syntheticpeptide"
EIFPGGGSTIYNENFRD

SEQ ID NO: 25 - protein, 17 aa, synthetic construct
  REGION 1..17: note = source = /note="Description of Artificial Sequence: Syntheticpeptide"
AIWPENADSVYNQKFKG

SEQ ID NO: 26 - protein, 17 aa, synthetic construct
  REGION 1..17: note = source = /note="Description of Artificial Sequence: Syntheticpeptide"
RIDPANGNTKYDPKFQG

SEQ ID NO: 27 - protein, 17 aa, synthetic construct
  REGION 1..17: note = source = /note="Description of Artificial Sequence: Syntheticpeptide"
EILPGSDSTKYVEKFKV

SEQ ID NO: 28 - protein, 17 aa, synthetic construct
  REGION 1..17: note = source = /note="Description of Artificial Sequence: Syntheticpeptide"
EISPDSSTINYTPSLKD

SEQ ID NO: 29 - protein, 17 aa, synthetic construct
  REGION 1..17: note = source = /note="Description of Artificial Sequence: Syntheticpeptide"
WIDTDTGEATYTDDFKG

SEQ ID NO: 30 - protein, 16 aa, synthetic construct
  REGION 1..16: note = source = /note="Description of Artificial Sequence: Syntheticpeptide"
HIWWDDDKRYNPALKS

SEQ ID NO: 31 - protein, 16 aa, synthetic construct
  REGION 1..16: note = source = /note="Description of Artificial Sequence: Syntheticpeptide"
VIWSGGSTDYNAAFIS

SEQ ID NO: 32 - protein, 9 aa, synthetic construct
  REGION 1..9: note = source = /note="Description of Artificial Sequence: Syntheticpeptide"
GGDGYALDY

SEQ ID NO: 33 - protein, 7 aa, synthetic construct
  REGION 1..7: note = source = /note="Description of Artificial Sequence: Syntheticpeptide"
FTTVFAY

SEQ ID NO: 34 - protein, 7 aa, synthetic construct
  REGION 1..7: note = source = /note="Description of Artificial Sequence: Syntheticpeptide"
THDWFDY

SEQ ID NO: 35 - protein, 11 aa, synthetic construct
  REGION 1..11: note = source = /note="Description of Artificial Sequence: Syntheticpeptide"
RALGNGYALGY

SEQ ID NO: 36 - protein, 9 aa, synthetic construct
  REGION 1..9: note = source = /note="Description of Artificial Sequence: Syntheticpeptide"
GTSYSWFAY

SEQ ID NO: 37 - protein, 15 aa, synthetic construct
  REGION 1..15: note = source = /note="Description of Artificial Sequence: Syntheticpeptide"
LGVMVYGSSPFWFAY

SEQ ID NO: 38 - protein, 11 aa, synthetic construct
  REGION 1..11: note = source = /note="Description of Artificial Sequence: Syntheticpeptide"
RALGNGYAMDY

SEQ ID NO: 39 - protein, 5 aa, synthetic construct
  REGION 1..5: note = source = /note="Description of Artificial Sequence: Syntheticpeptide"
KTTNY

SEQ ID NO: 40 - protein, 11 aa, synthetic construct
  REGION 1..11: note = source = /note="Description of Artificial Sequence: Syntheticpeptide"
RGYYDAAWFDY

SEQ ID NO: 41 - protein, 5 aa, synthetic construct
  REGION 1..5: note = source = /note="Description of Artificial Sequence: Syntheticpeptide"
EGGNY

SEQ ID NO: 42 - protein, 9 aa, synthetic construct
  REGION 1..9: note = source = /note="Description of Artificial Sequence: Syntheticpeptide"
SGNYGAMDY

SEQ ID NO: 43 - protein, 11 aa, synthetic construct
  REGION 1..11: note = source = /note="Description of Artificial Sequence: Syntheticpeptide"
GGYHYPGWLVY

SEQ ID NO: 44 - protein, 7 aa, synthetic construct
  REGION 1..7: note = source = /note="Description of Artificial Sequence: Syntheticpeptide"
PSPALDY

SEQ ID NO: 45 - protein, 10 aa, synthetic construct
  REGION 1..10: note = source = /note="Description of Artificial Sequence: Syntheticpeptide"
EEYGLFGFPY

SEQ ID NO: 46 - protein, 14 aa, synthetic construct
  REGION 1..14: note = source = /note="Description of Artificial Sequence: Syntheticpeptide"
IDGIYDGSFYAMDY

SEQ ID NO: 47 - protein, 12 aa, synthetic construct
  REGION 1..12: note = source = /note="Description of Artificial Sequence: Syntheticpeptide"
DYGSTYVDAIDY

SEQ ID NO: 48 - protein, 11 aa, synthetic construct
  REGION 1..11: note = source = /note="Description of Artificial Sequence: Syntheticpeptide"
SASQVISNYLN

SEQ ID NO: 49 - protein, 10 aa, synthetic construct
  REGION 1..10: note = source = /note="Description of Artificial Sequence: Syntheticpeptide"
SASSSGRYTF

SEQ ID NO: 50 - protein, 11 aa, synthetic construct
  REGION 1..11: note = source = /note="Description of Artificial Sequence: Syntheticpeptide"
RASQDISNYFN

SEQ ID NO: 51 - protein, 11 aa, synthetic construct
  REGION 1..11: note = source = /note="Description of Artificial Sequence: Syntheticpeptide"
KASDHINNWLA

SEQ ID NO: 52 - protein, 16 aa, synthetic construct
  REGION 1..16: note = source = /note="Description of Artificial Sequence: Syntheticpeptide"
RSSQNIVHSDGNTYLE

SEQ ID NO: 53 - protein, 11 aa, synthetic construct
  REGION 1..11: note = source = /note="Description of Artificial Sequence: Syntheticpeptide"
KASQFVSDAVA

SEQ ID NO: 54 - protein, 11 aa, synthetic construct
  REGION 1..11: note = source = /note="Description of Artificial Sequence: Syntheticpeptide"
RASQEISGYLS

SEQ ID NO: 55 - protein, 12 aa, synthetic construct
  REGION 1..12: note = source = /note="Description of Artificial Sequence: Syntheticpeptide"
SASSSLSSSYLY

SEQ ID NO: 56 - protein, 17 aa, synthetic construct
  REGION 1..17: note = source = /note="Description of Artificial Sequence: Syntheticpeptide"
KSSQSLLNSGNQKNSLA

SEQ ID NO: 57 - protein, 10 aa, synthetic construct
  REGION 1..10: note = source = /note="Description of Artificial Sequence: Syntheticpeptide"
RASSSVNHMY

SEQ ID NO: 58 - protein, 11 aa, synthetic construct
  REGION 1..11: note = source = /note="Description of Artificial Sequence: Syntheticpeptide"
KASQNVDSYVA

SEQ ID NO: 59 - protein, 11 aa, synthetic construct
  REGION 1..11: note = source = /note="Description of Artificial Sequence: Syntheticpeptide"
RASQSISDYVY

SEQ ID NO: 60 - protein, 11 aa, synthetic construct
  REGION 1..11: note = source = /note="Description of Artificial Sequence: Syntheticpeptide"
KASEDIYNRLA

SEQ ID NO: 61 - protein, 15 aa, synthetic construct
  REGION 1..15: note = source = /note="Description of Artificial Sequence: Syntheticpeptide"
RASESVDSYGNSFMH

SEQ ID NO: 62 - protein, 15 aa, synthetic construct
  REGION 1..15: note = source = /note="Description of Artificial Sequence: Syntheticpeptide"
RASESVESYGNRYMT

SEQ ID NO: 63 - protein, 7 aa, synthetic construct
  REGION 1..7: note = source = /note="Description of Artificial Sequence: Syntheticpeptide"
FTSSLRS

SEQ ID NO: 64 - protein, 7 aa, synthetic construct
  REGION 1..7: note = source = /note="Description of Artificial Sequence: Syntheticpeptide"
DTSKLAS

SEQ ID NO: 65 - protein, 7 aa, synthetic construct
  REGION 1..7: note = source = /note="Description of Artificial Sequence: Syntheticpeptide"
YTSRLQS

SEQ ID NO: 66 - protein, 7 aa, synthetic construct
  REGION 1..7: note = source = /note="Description of Artificial Sequence: Syntheticpeptide"
GTTNLET

SEQ ID NO: 67 - protein, 7 aa, synthetic construct
  REGION 1..7: note = source = /note="Description of Artificial Sequence: Syntheticpeptide"
KVSNRFS

SEQ ID NO: 68 - protein, 7 aa, synthetic construct
  REGION 1..7: note = source = /note="Description of Artificial Sequence: Syntheticpeptide"
SASYRYT

SEQ ID NO: 69 - protein, 7 aa, synthetic construct
  REGION 1..7: note = source = /note="Description of Artificial Sequence: Syntheticpeptide"
GASNLET

SEQ ID NO: 70 - protein, 7 aa, synthetic construct
  REGION 1..7: note = source = /note="Description of Artificial Sequence: Syntheticpeptide"
AASTLDS

SEQ ID NO: 71 - protein, 7 aa, synthetic construct
  REGION 1..7: note = source = /note="Description of Artificial Sequence: Syntheticpeptide"
GASNLAS

SEQ ID NO: 72 - protein, 7 aa, synthetic construct
  REGION 1..7: note = source = /note="Description of Artificial Sequence: Syntheticpeptide"
LASTRES

SEQ ID NO: 73 - protein, 7 aa, synthetic construct
  REGION 1..7: note = source = /note="Description of Artificial Sequence: Syntheticpeptide"
YTSTLAP

SEQ ID NO: 74 - protein, 7 aa, synthetic construct
  REGION 1..7: note = source = /note="Description of Artificial Sequence: Syntheticpeptide"
SASYRFS

SEQ ID NO: 75 - protein, 7 aa, synthetic construct
  REGION 1..7: note = source = /note="Description of Artificial Sequence: Syntheticpeptide"
YASQSIS

SEQ ID NO: 76 - protein, 7 aa, synthetic construct
  REGION 1..7: note = source = /note="Description of Artificial Sequence: Syntheticpeptide"
AATSLET

SEQ ID NO: 77 - protein, 7 aa, synthetic construct
  REGION 1..7: note = source = /note="Description of Artificial Sequence: Syntheticpeptide"
RASNLES

SEQ ID NO: 78 - protein, 7 aa, synthetic construct
  REGION 1..7: note = source = /note="Description of Artificial Sequence: Syntheticpeptide"
RAANLQS

SEQ ID NO: 79 - protein, 9 aa, synthetic construct
  REGION 1..9: note = source = /note="Description of Artificial Sequence: Syntheticpeptide"
QQYSKLPWT

SEQ ID NO: 80 - protein, 9 aa, synthetic construct
  REGION 1..9: note = source = /note="Description of Artificial Sequence: Syntheticpeptide"
FQGTGYPLT

SEQ ID NO: 81 - protein, 9 aa, synthetic construct
  REGION 1..9: note = source = /note="Description of Artificial Sequence: Syntheticpeptide"
HQVRTLPWT

SEQ ID NO: 82 - protein, 9 aa, synthetic construct
  REGION 1..9: note = source = /note="Description of Artificial Sequence: Syntheticpeptide"
QQYWNTPFT

SEQ ID NO: 83 - protein, 8 aa, synthetic construct
  REGION 1..8: note = source = /note="Description of Artificial Sequence: Syntheticpeptide"
FQGSHVLT

SEQ ID NO: 84 - protein, 9 aa, synthetic construct
  REGION 1..9: note = source = /note="Description of Artificial Sequence: Syntheticpeptide"
QQHYIVPYT

SEQ ID NO: 85 - protein, 9 aa, synthetic construct
  REGION 1..9: note = source = /note="Description of Artificial Sequence: Syntheticpeptide"
LQYGSYPWT

SEQ ID NO: 86 - protein, 9 aa, synthetic construct
  REGION 1..9: note = source = /note="Description of Artificial Sequence: Syntheticpeptide"
HQWSSYPLT

SEQ ID NO: 87 - protein, 9 aa, synthetic construct
  REGION 1..9: note = source = /note="Description of Artificial Sequence: Syntheticpeptide"
QQHHSTPYT

SEQ ID NO: 88 - protein, 11 aa, synthetic construct
  REGION 1..11: note = source = /note="Description of Artificial Sequence: Syntheticpeptide"
QQFTISPSMYT

SEQ ID NO: 89 - protein, 9 aa, synthetic construct
  REGION 1..9: note = source = /note="Description of Artificial Sequence: Syntheticpeptide"
QQYNISPYT

SEQ ID NO: 90 - protein, 9 aa, synthetic construct
  REGION 1..9: note = source = /note="Description of Artificial Sequence: Syntheticpeptide"
QNGHNFPYT

SEQ ID NO: 91 - protein, 9 aa, synthetic construct
  REGION 1..9: note = source = /note="Description of Artificial Sequence: Syntheticpeptide"
QQYWSNPLT

SEQ ID NO: 92 - protein, 8 aa, synthetic construct
  REGION 1..8: note = source = /note="Description of Artificial Sequence: Syntheticpeptide"
QQSNEDYT

SEQ ID NO: 93 - protein, 9 aa, synthetic construct
  REGION 1..9: note = source = /note="Description of Artificial Sequence: Syntheticpeptide"
QQSNEDPWT

SEQ ID NO: 94 - protein, 118 aa, synthetic construct
  REGION 1..118: note = source = /note="Description of Artificial Sequence: Syntheticpolypeptide"
EVQLVESGGGLVKPGGSLKLSCAPSGFTFSSYGISWVRQTPEKRLEWVATVSSGGRYTYYPDSVKGRFTISRDNAENTLYLQMSSLRSEDTAMYYCTRGGDGYALDYWGQGTSVTVSS

SEQ ID NO: 95 - protein, 116 aa, synthetic construct
  REGION 1..116: note = source = /note="Description of Artificial Sequence: Syntheticpolypeptide"
EVQLQQSGAELVRPGALVNLSCKASGFNIKDYYMNWVKQRPEQGLEWTGWIDPENDDTIYDPKFQGKATITADTSSNTVYLQLTSLTSEDTAVYYCAAFTTVFAYWGHQTMVTVSA

SEQ ID NO: 96 - protein, 115 aa, synthetic construct
  REGION 1..115: note = source = /note="Description of Artificial Sequence: Syntheticpolypeptide"
QVQVKESGPGLVAPSQSLSITCTVSGFSLTNYGVSWIRQPPGKGLEWLGVIWGDGSINYHSALISRLTITKDNSKSQVFLKLNSLEADDTATYYCAKTHDWFDYWGQGTLVTVSA

SEQ ID NO: 97 - protein, 120 aa, synthetic construct
  REGION 1..120: note = source = /note="Description of Artificial Sequence: Syntheticpolypeptide"
EVQLQQSGAELVKPGASVKLSCTAADFNIKDTYMHWVKQRPEQGLEWIGRIDPSNGNAKYDPKFQGKASITADSSSNTAYLHLSSLTSEDTAVYYCASRALGNGYALGYWGQGTSVTVSS

SEQ ID NO: 98 - protein, 118 aa, synthetic construct
  REGION 1..118: note = source = /note="Description of Artificial Sequence: Syntheticpolypeptide"
EVQLQQSGAELVKPGASVKLSCTASDFNIIDTYIHWVKQRPEQGLEWIGRIDPANGNTKYDPKFQDKAALTSDTDSNTAYLLFNSLTSEDTAVYYCARGTSYSWFAYWGQGTLVSVSA

SEQ ID NO: 99 - protein, 124 aa, synthetic construct
  REGION 1..124: note = source = /note="Description of Artificial Sequence: Syntheticpolypeptide"
QVQLQQPGAEIVKPGASVRLSCKASGYSFTSYWIHWVKQRPGQGLEWIGEIDPSVSNSNYNQKFKGKATLTADKSSSTAYMQLSGLTSEDSAVYFCVRLGVMVYGSSPFWFAYWGQGTLVTVSA

SEQ ID NO: 100 - protein, 124 aa, synthetic construct; identical to SEQ ID NO: 99
  REGION 1..124: note = source = /note="Description of Artificial Sequence: Syntheticpolypeptide"

SEQ ID NO: 101 - protein, 120 aa, synthetic construct
  REGION 1..120: note = source = /note="Description of Artificial Sequence: Syntheticpolypeptide"
EVQLQQSGAELLKPGASVRLSCTASGFNIQDTFTHWVRQRPEQGLEWIGRIDPSNGNTKYDPKFQGKAKILADTSSNTAYLQLIGLTSEDTAVYYCASRALGNGYAMDYWGQGTSVTVSS

SEQ ID NO: 102 - protein, 114 aa, synthetic construct
  REGION 1..114: note = source = /note="Description of Artificial Sequence: Syntheticpolypeptide"
EVPLQQSGPELVKPGATVKISCKPSGDTFTEYTMNWVRQSHGKSLEWIGGINPNNGETSYNQKFKGKATLTVDKSSSTAFMDLRILTSEDSAVYFCARKTTNYWGQGTTLIVSS

SEQ ID NO: 103 - protein, 120 aa, synthetic construct
  REGION 1..120: note = source = /note="Description of Artificial Sequence: Syntheticpolypeptide"
QIQLQQSGAELMKPGASVRMSCKASGYTFSSYWIEWVKQRSGHGLEWIGEIFPGGGSTIYNENFRDKATFTADTSSNTAYMQLSSLTSEDSAVYFCARRGYYDAAWFDYWGQGTLVTVSA

SEQ ID NO: 104 - protein, 114 aa, synthetic construct
  REGION 1..114: note = source = /note="Description of Artificial Sequence: Syntheticpolypeptide"
QVQLKQSGAELVRPGTSVTLSCKASGYTFTDYEMHWMKQTPVYGLEWIGAIWPENADSVYNQKFKGKVTLTADKSSSTAYMDLRSLTSEDSAVYYCTREGGNYWGQGTTLTVSS

SEQ ID NO: 105 - protein, 118 aa, synthetic construct
  REGION 1..118: note = source = /note="Description of Artificial Sequence: Syntheticpolypeptide"
EVQLQQSGTELVRPGASVKLSCTSSDFNIKDTYIHWVKQRPEQGLDWLGRIDPANGNTKYDPKFQGKAAMTSDTSSNTAYLRLSSLTSEDTAVYYCASSGNYGAMDYWGQGTSVTVSS

SEQ ID NO: 106 - protein, 120 aa, synthetic construct
  REGION 1..120: note = source = /note="Description of Artificial Sequence: Syntheticpolypeptide"
QVQLQQSGDELMKPGASVKISCKVTGNTFSSYWIEWVKQRPGHGLEWIGEILPGSDSTKYVEKFKVKATFTADTSSNTAYMQLSSLTSEDSAVYYCARGGYHYPGWLVYWGQGTLVTVSA

SEQ ID NO: 107 - protein, 116 aa, synthetic construct
  REGION 1..116: note = source = /note="Description of Artificial Sequence: Syntheticpolypeptide"
EVKFLESGGGLVQPGGSLRLSCAVSGIDFSRYWMSWVRQAPGKGLEWIGEISPDSSTINYTPSLKDKFVISRDNAKNTLYLQMSKVRSADTALYYCARPSPALDYWGQGTLVTVSA

SEQ ID NO: 108 - protein, 119 aa, synthetic construct
  REGION 1..119: note = source = /note="Description of Artificial Sequence: Syntheticpolypeptide"
QIQLVQSGPELKKPGETAKISCKASGYAFSNYGMNWVKQAPGKDLKWMGWIDTDTGEATYTDDFKGRFVFSLETSASTAYLQINNLKNEDMATYFCAREEYGLFGFPYWGHGTLVTVSA

SEQ ID NO: 109 - protein, 124 aa, synthetic construct
  REGION 1..124: note = source = /note="Description of Artificial Sequence: Syntheticpolypeptide"
QVTLKESGPGILQPSQTLSLTCSFSGFSLSTSAMGIGWIRQPSGKGLEWLAHIWWDDDKRYNPALKSRLTISKDTSRNQVFLKIASVDTADTATYFCARIDGIYDGSFYAMDYWGQGTSVTVSS

SEQ ID NO: 110 - protein, 120 aa, synthetic construct
  REGION 1..120: note = source = /note="Description of Artificial Sequence: Syntheticpolypeptide"
QVQLKQSGPGLVQPSQSLSVACTVSDFSLTTYGVHWVRQSPGKGLEWLGVIWSGGSTDYNAAFISRLTISKDNSKSQVFFKMNSLQTTDTAIYYCARDYGSTYVDAIDYWGQGTSVTVSS

SEQ ID NO: 111 - protein, 107 aa, synthetic construct
  REGION 1..107: note = source = /note="Description of Artificial Sequence: Syntheticpolypeptide"
DIQMTQTTSSLSASLGDRVTIICSASQVISNYLNWYQQKPDGTVKLLIYFTSSLRSGVPSRFSGSGSGTDYSLTISNLEPEDVATYFCQQYSKLPWTFGGGTKLELK

SEQ ID NO: 112 - protein, 106 aa, synthetic construct
  REGION 1..106: note = source = /note="Description of Artificial Sequence: Syntheticpolypeptide"
ENVLTQSPAIMSASPGEKVTMTCSASSSGRYTFWYQQKSNTAPKLWIYDTSKLASGVPGRFSGSGSGNSYSLTISSMEAEDVATYYCFQGTGYPLTFGAGTKLELK

SEQ ID NO: 113 - protein, 107 aa, synthetic construct
  REGION 1..107: note = source = /note="Description of Artificial Sequence: Syntheticpolypeptide"
DIQMTQTPSSLSASLGDRVTINCRASQDISNYFNWYQQKPNGTIKLLIYYTSRLQSGVPSRFSGSGSGTDYSLTISNLEQEDKATYFCHQVRTLPWTFGGGTKLEIK

SEQ ID NO: 114 - protein, 107 aa, synthetic construct
  REGION 1..107: note = source = /note="Description of Artificial Sequence: Syntheticpolypeptide"
DIQMTQSSSYLSVSLGGSVTITCKASDHINNWLAWYQQKPGNAPRLLIYGTTNLETGVPSRFSGSGSGRDYILSITSLQSEDVASYYCQQYWNTPFTFGSGTKLEIK

SEQ ID NO: 115 - protein, 111 aa, synthetic construct
  REGION 1..111: note = source = /note="Description of Artificial Sequence: Syntheticpolypeptide"
AVLMTQTPLSLPVSLGDQASISCRSSQNIVHSDGNTYLEWYLQKPGQSPKLLIYKVSNRFSGVPDRFSGSGSGRDFTLKISRVEAGDLGVYYCFQGSHVLTFGAGTRLELK

SEQ ID NO: 116 - protein, 107 aa, synthetic construct
  REGION 1..107: note = source = /note="Description of Artificial Sequence: Syntheticpolypeptide"
DIVMTQSQKFMSTSVGDRVSITCKASQFVSDAVAWYQQKPGQSPKLLICSASYRYTGVPDRFTGSGSGTDFTFTISSVRTEDLAVYYCQQHYIVPYTFGGGTTLEIE

SEQ ID NO: 117 - protein, 107 aa, synthetic construct; identical to SEQ ID NO: 116
  REGION 1..107: note = source = /note="Description of Artificial Sequence: Syntheticpolypeptide"

SEQ ID NO: 118 - protein, 107 aa, synthetic construct
  REGION 1..107: note = source = /note="Description of Artificial Sequence: Syntheticpolypeptide"
DIQMTQSSSYLSVSLGGRVTITCKASDHINNWLAWYQQKPGNAPRLLISGASNLETGIPSRFSGSGSGKDYTLTITSLQTEDVATYYCQQYWNTPFTFGSGTKLEIK

SEQ ID NO: 119 - protein, 107 aa, synthetic construct
  REGION 1..107: note = source = /note="Description of Artificial Sequence: Syntheticpolypeptide"
DIQMTQSPSSLSASLGERVSLTCRASQEISGYLSWLQQKPDGTIKRLIYAASTLDSGVPRRFSGSRSGSDYSLTISSLESEDFADYYCLQYGSYPWTFGGGTKLELK

SEQ ID NO: 120 - protein, 108 aa, synthetic construct
  REGION 1..108: note = source = /note="Description of Artificial Sequence: Syntheticpolypeptide"
QIVLTQSPAIMSASPGERVTLTCSASSSLSSSYLYWYQQKPGSSPKLWIYGASNLASGVPGRFSGSGSGTSYSLTISSMEAEDAASYFCHQWSSYPLTFGSGTKLELK

SEQ ID NO: 121 - protein, 113 aa, synthetic construct
  REGION 1..113: note = source = /note="Description of Artificial Sequence: Syntheticpolypeptide"
DIVMTQSPSSLPMSVGQKVTMSCKSSQSLLNSGNQKNSLAWYQQKPGQSPKLLVYLASTRESGVPDRFIGSGSGTDFTLTISSVQAEDLADYFCQQHHSTPYTFGGGTKLELK

SEQ ID NO: 122 - protein, 108 aa, synthetic construct
  REGION 1..108: note = source = /note="Description of Artificial Sequence: Syntheticpolypeptide"
ESVLTQSPALMSASLGEKVTMTCRASSSVNHMYWYQQKSDASPKLWIYYTSTLAPGVPARFSGSGSGNSYSLTISSMEGEDAATYYCQQFTISPSMYTFGGGTKLEIK

SEQ ID NO: 123 - protein, 107 aa, synthetic construct
  REGION 1..107: note = source = /note="Description of Artificial Sequence: Syntheticpolypeptide"
DIVMTQSQKFMSTSVGDRVSVTCKASQNVDSYVAWYQQKAGQSPKPLIYSASYRFSGVPDRFTGSGSGTEFTLTISNVQSEDLAEYFCQQYNISPYTFGGGTKLEIK

SEQ ID NO: 124 - protein, 107 aa, synthetic construct
  REGION 1..107: note = source = /note="Description of Artificial Sequence: Syntheticpolypeptide"
DIVMTQSPATLSVTPGDRVSLSCRASQSISDYVYWYQQKSHESPRLLIIYASQSISGIPSRFSGSGSGSDFTLSINSVEPEDVGVYYCQNGHNFPYTFGGGTKLEIK

SEQ ID NO: 125 - protein, 107 aa, synthetic construct
  REGION 1..107: note = source = /note="Description of Artificial Sequence: Syntheticpolypeptide"
DIQMTQSSSSFSVSLGDRVTITCKASEDIYNRLAWYQQKPGSAPRLLISAATSLETGVPSRFSGSGSGKDYTLSITSLQTEDVATYYCQQYWSNPLTFGAGTKLEIK

SEQ ID NO: 126 - protein, 110 aa, synthetic construct
  REGION 1..110: note = source = /note="Description of Artificial Sequence: Syntheticpolypeptide"
DIVLTQSPASLAVSLGQRATISCRASESVDSYGNSFMHWYQQKPGQPPKLLIYRASNLESGIPARFSGSGSRTDFTLTINPVEADDVANYYCQQSNEDYTFGGGTKLEIK

SEQ ID NO: 127 - protein, 111 aa, synthetic construct
  REGION 1..111: note = source = /note="Description of Artificial Sequence: Syntheticpolypeptide"
DIVLTQSPTSLAVSLGQRATISCRASESVESYGNRYMTWYQQKPGQPPKLLIYRAANLQSGIPARFSGSGSRTDFTLTIDPVEADDVATYYCQQSNEDPWTFGGGTKVEIK

SEQ ID NO: 128 - protein, 120 aa, synthetic construct
  REGION 1..120: note = source = /note="Description of Artificial Sequence: Syntheticpolypeptide"
EVQLVESGGGLVQPGGSLRLSCAASDFSLTTYGVHWVRQAPGKGLEWLGVIWSGGSTDYNAAFISRLTISKDNSKNTVYLQMNSLRAEDTAVYYCARDYGSTYVDAIDYWGQGTLVTVSS

SEQ ID NO: 129 - protein, 450 aa, synthetic construct
  REGION 1..450: note = source = /note="Description of Artificial Sequence: Syntheticpolypeptide"
EVQLVESGGGLVQPGGSLRLSCAASDFSLTTYGVHWVRQAPGKGLEWLGVIWSGGSTDYNAAFISRLTISKDNSKNTVYLQMNSLRAEDTAVYYCARDYGSTYVDAIDYWGQGTLVTVSSASTKGPSVFPLAPSSKSTSGGTAALGCLVKDYFPEPVTVSWNSGALTSGVHTFPAVLQSSGLYSLSSVVTVPSSSLGTQTYICNVNHKPSNTKVDKKVEPKSCDKTHTCPPCPAPELLGGPSVFLFPPKPKDTLMISRTPEVTCVVVDVSHEDPEVKFNWYVDGVEVHNAKTKPREEQYGSTYRVVSVLTVLHQDWLNGKEYKCKVSNKALPAPIEKTISKAKGQPREPQVYTLPPSREEMTKNQVSLSCAVKGFYPSDIAVEWESNGQPENNYKTTPPVLDSDGSFFLVSKLTVDKSRWQQGNVFSCSVMHEALHNHYTQKSLSLSPGK

SEQ ID NO: 130 - protein, 111 aa, synthetic construct
  REGION 1..111: note = source = /note="Description of Artificial Sequence: Syntheticpolypeptide"
DIVLTQSPDSLAVSLGERATINCRASESVESYGNRYMTWYQQKPGQPPKLLIYRAANLQSGVPDRFSGSGSGTDFTLTISSLQAEDVAVYYCQQSNEDPWTFGQGTKVEIK

SEQ ID NO: 131 - protein, 218 aa, synthetic construct
  REGION 1..218: note = source = /note="Description of Artificial Sequence: Syntheticpolypeptide"
DIVLTQSPDSLAVSLGERATINCRASESVESYGNRYMTWYQQKPGQPPKLLIYRAANLQSGVPDRFSGSGSGTDFTLTISSLQAEDVAVYYCQQSNEDPWTFGQGTKVEIKRTVAAPSVFIFPPSDEQLKSGTASVVCLLNNFYPREAKVQWKVDNALQSGNSQESVTEQDSKDSTYSLSSTLTLSKADYEKHKVYACEVTHQGLSSPVTKSFNRGEC

SEQ ID NO: 132 - protein, 116 aa, synthetic construct
  REGION 1..116: note = source = /note="Description of Artificial Sequence: Syntheticpolypeptide"
EVQLVESGGGLVQPGGSLRLSCAASGFTFTSNYISWVRQAPGKGLEWVGEIDPYDGDTYYADSVKGRFTISADTSKNTAYLQMNSLRAEDTAVYYCATGTDVMDYWGQGTLVTVSS

SEQ ID NO: 133 - protein, 446 aa, synthetic construct
  REGION 1..446: note = source = /note="Description of Artificial Sequence: Syntheticpolypeptide"
EVQLVESGGGLVQPGGSLRLSCAASGFTFTSNYISWVRQAPGKGLEWVGEIDPYDGDTYYADSVKGRFTISADTSKNTAYLQMNSLRAEDTAVYYCATGTDVMDYWGQGTLVTVSSASTKGPSVFPLAPSSKSTSGGTAALGCLVKDYFPEPVTVSWNSGALTSGVHTFPAVLQSSGLYSLSSVVTVPSSSLGTQTYICNVNHKPSNTKVDKKVEPKSCDKTHTCPPCPAPELLGGPSVFLFPPKPKDTLMISRTPEVTCVVVDVSHEDPEVKFNWYVDGVEVHNAKTKPREEQYGSTYRVVSVLTVLHQDWLNGKEYKCKVSNKALPAPIEKTISKAKGQPREPQVYTLPPSREEMTKNQVSLWCLVKGFYPSDIAVEWESNGQPENNYKTTPPVLDSDGSFFLYSKLTVDKSRWQQGNVFSCSVMHEALHNHYTQKSLSLSPGK

SEQ ID NO: 134 - protein, 107 aa, synthetic construct
  REGION 1..107: note = source = /note="Description of Artificial Sequence: Syntheticpolypeptide"
DIQMTQSPSSLSASVGDRVTITCRASQDVSTAVAWYQQKPGKAPKLLIYSASFLYSGVPSRFSGSGSGTDFTLTISSLQPEDFATYYCQQSYTTPPTFGQGTKVEIK

SEQ ID NO: 135 - protein, 214 aa, synthetic construct
  REGION 1..214: note = source = /note="Description of Artificial Sequence: Syntheticpolypeptide"
DIQMTQSPSSLSASVGDRVTITCRASQDVSTAVAWYQQKPGKAPKLLIYSASFLYSGVPSRFSGSGSGTDFTLTISSLQPEDFATYYCQQSYTTPPTFGQGTKVEIKRTVAAPSVFIFPPSDEQLKSGTASVVCLLNNFYPREAKVQWKVDNALQSGNSQESVTEQDSKDSTYSLSSTLTLSKADYEKHKVYACEVTHQGLSSPVTKSFNRGEC

SEQ ID NO: 136 - protein, 5 aa, synthetic construct
  REGION 1..5: note = source = /note="Description of Artificial Sequence: Syntheticpeptide"
SNYIS

SEQ ID NO: 137 - protein, 17 aa, synthetic construct
  REGION 1..17: note = source = /note="Description of Artificial Sequence: Syntheticpeptide"
EIDPYDGDTYYADSVKG

SEQ ID NO: 138 - protein, 7 aa, synthetic construct
  REGION 1..7: note = source = /note="Description of Artificial Sequence: Syntheticpeptide"
GTDVMDY

SEQ ID NO: 139 - protein, 11 aa, synthetic construct
  REGION 1..11: note = source = /note="Description of Artificial Sequence: Syntheticpeptide"
RASQDVSTAVA

SEQ ID NO: 140 - protein, 7 aa, synthetic construct
  REGION 1..7: note = source = /note="Description of Artificial Sequence: Syntheticpeptide"
SASFLYS

SEQ ID NO: 141 - protein, 9 aa, synthetic construct
  REGION 1..9: note = source = /note="Description of Artificial Sequence: Syntheticpeptide"
QQSYTTPPT

SEQ ID NO: 142 - protein, 34 aa, unidentified
  REGION 1..34: note = source = /note="Description of Unknown: beta-Klothopeptide"
SSPTRLAVIPWGVRKLLRWVRRNYGDMDIYITAS

SEQ ID NO: 143 - protein, 16 aa, unidentified
  REGION 1..16: note = source = /note="Description of Unknown: Fibroblast Growth FactorReceptor 1 peptide"
KLHAVPAAKTVKFKCP

SEQ ID NO: 144 - protein, 14 aa, unidentified
  REGION 1..14: note = source = /note="Description of Unknown: Fibroblast Growth FactorReceptor 1 peptide"
FKPDHRIGGYKVRY

SEQ ID NO: 145 - protein, 992 aa, Homo sapiens
FSGDGRAIWSKNPNFTPVNESQLFLYDTFPKNFFWGIGTGALQVEGSWKKDGKGPSIWDHFIHTHLKNVSSTNGSSDSYIFLEKDLSALDFIGVSFYQFSISWPRLFPDGIVTVANAKGLQYYSTLLDALVLRNIEPIVTLYHWDLPLALQEKYGGWKNDTIIDIFNDYATYCFQMFGDRVKYWITIHNPYLVAWHGYGTGMHAPGEKGNLAAVYTVGHNLIKAHSKVWHNYNTHFRPHQKGWLSITLGSHWIEPNRSENTMDIFKCQQSMVSVLGWFANPIHGDGDYPEGMRKKLFSVLPIFSEAEKHEMRGTADFFAFSFGPNNFKPLNTMAKMGQNVSLNLREALNWIKLEYNNPRILIAENGWFTDSRVKTEDTTAIYMMKNFLSQVLQAIRLDEIRVFGYTAWSLLDGFEWQDAYTIRRGLFYVDFNSKQKERKPKSSAHYYKQIIRENGFSLKESTPDVQGQFPCDFSWGVTESVLKPESVASSPQFSDPHLYVWNATGNRLLHRVEGVRLKTRPAQCTDFVNIKKQLEMLARMKVTHYRFALDWASVLPTGNLSAVNRQALRYYRCVVSEGLKLGISAMVTLYYPTHAHLGLPEPLLHADGWLNPSTAEAFQAYAGLCFQELGDLVKLWITINEPNRLSDIYNRSGNDTYGAAHNLLVAHALAWRLYDRQFRPSQRGAVSLSLHADWAEPANPYADSHWRAAERFLQFEIAWFAEPLFKTGDYPAAMREYIASKHRRGLSSSALPRLTEAERRLLKGTVDFCALNHFTTRFVMHEQLAGSRYDSDRDIQFLQDITRLSSPTRLAVIPWGVRKLLRWVRRNYGDMDIYITASGIDDQALEDDRLRKYYLGKYLQEVLKAYLIDKVRIKGYYAFKLAEEKSKPRFGFFTSDFKAKSSIQFYNKVISSRGFPFENSSSRCSQTQENTECTVCLFLVQKKPLIFLGCCFFSTLVLLLSIAIFQRQKRRKFWKAKNLQHIPLKKGKRVVS

SEQ ID NO: 146 - protein, 820 aa, Homo sapiens
MWSWKCLLFWAVLVTATLCTARPSPTLPEQAQPWGAPVEVESFLVHPGDLLQLRCRLRDDVQSINWLRDGVQLAESNRTRITGEEVEVQDSVPADSGLYACVTSSPSGSDTTYFSVNVSDALPSSEDDDDDDDSSSEEKETDNTKPNPVAPYWTSPEKMEKKLHAVPAAKTVKFKCPSSGTPNPTLRWLKNGKEFKPDHRIGGYKVRYATWSIIMDSVVPSDKGNYTCIVENEYGSINHTYQLDVVERSPHRPILQAGLPANKTVALGSNVEFMCKVYSDPQPHIQWLKHIEVNGSKIGPDNLPYVQILKTAGVNTTDKEMEVLHLRNVSFEDAGEYTCLAGNSIGLSHHSAWLTVLEALEERPAVMTSPLYLEIIIYCTGAFLISCMVGSVIVYKMKSGTKKSDFHSQMAVHKLAKSIPLRRQVTVSADSSASMNSGVLLVRPSRLSSSGTPMLAGVSEYELPEDPRWELPRDRLVLGKPLGEGCFGQVVLAEAIGLDKDKPNRVTKVAVKMLKSDATEKDLSDLISEMEMMKMIGKHKNIINLLGACTQDGPLYVIVEYASKGNLREYLQARRPPGLEYCYNPSHNPEEQLSSKDLVSCAYQVARGMEYLASKKCIHRDLAARNVLVTEDNVMKIADFGLARDIHHIDYYKKTTNGRLPVKWMAPEALFDRIYTHQSDVWSFGVLLWEIFTLGGSPYPGVPVEELFKLLKEGHRMDKPSNCTNELYMMMRDCWHAVPSQRPTFKQLVEDLDRIVALTSNQEYLDLSMPLDQYSPSFPDTRSSTCSSGEDSVFSHEPLPEEPCLPRHPAQLANGGLKRR

SEQ ID NO: 147 - protein, 948 aa, synthetic construct
  REGION 1..948: note = source = /note="Description of Artificial Sequence: Syntheticpolypeptide"
DYKDDDDKLEFSGDGKAIWDKKQYVSPVNPGQLFLYDTFPKNFSWGVGTGAFQVEGSWKADGRGPSIWDRYVDSHLRGVNSTDRSTDSYVFLEKDLLALDFLGVSFYQFSISWPRLFPNGTVAAVNAKGLQYYRALLDSLVLRNIEPIVTLYHWDLPLTLQEEYGGWKNATMIDLFNDYATYCFQTFGDRVKYWITIHNPYLVAWHGFGTGMHAPGEKGNLTAVYTVGHNLIKAHSKVWHNYDKNFRPHQKGWLSITLGSHWIEPNRTENMEDVINCQHSMSSVLGWFANPIHGDGDYPEFMKTSSVIPEFSEAEKEEVRGTADFFAFSFGPNNFRPSNTVVKMGQNVSLNLRQVLNWIKLEYDNPRILISENGWFTDSYIKTEDTTAIYMMKNFLNQVLQAIKFDEIQVFGYTAWTLLDGFEWQDAYTTRRGLFYVDFNSEQKERKPKSSAHYYKQIIQDNGFPLQESTPDMKGQFPCDFSWGVTESVLKPEFTVSSPQFTDPHLYVWNVTGNRLLYRVEGVRLKTRPSQCTDYVSIKKRVEMLAKMKVTHYQFALDWTSILPTGNLSKINRQVLRYYRCVVSEGLKLGISPMVTLYHPTHSHLGLPMPLLSSGGWLNTNTAKAFQDYAGLCFKELGDLVKLWITINEPNRLSDMYNRTSNDTYRAAHNLMIAHAQVWHLYDRQYRPVQHGAVSLSLHSDWAEPANPYVESHWKAAERFLQFEIAWFADPLFKTGDYPLAMKEYIASKKQRGLSSSVLPRFTLKESRLVKGTIDFYALNHFTTRFVIHKQLNTNCSVADRDVQFLQDITRLSSPSRLAVTPWGMRKLLGWIRRNYRDMDIYVTANGIDDLALEDDQIRKYYLEKYVQEALKAYLIDKVKIKGYYAFKLTEEKSKPRFGFFTSDFKAKSSVQFYSKLISSSGFSSENRSPACGQPPEDTECAICSFLT

SEQ ID NO: 148 - protein, 949 aa, synthetic construct
  REGION 1..949: note = source = /note="Description of Artificial Sequence: Syntheticpolypeptide"
DYKDDDDKLDFPGDGRAVWSQNPNLSPVNESQLFLYDTFPKNFFWGVGTGAFQVEGSWKKDGKGLSVWDHFIATHLNVSSRDGSSDSYIFLEKDLSALDFLGVSFYQFSISWPRLFPDGTVAVANAKGLQYYNRLLDSLLLRNIEPVVTLYHWDLPWALQEKYGGWKNETLIDLFNDYATYCFQTFGDRVKYWITIHNPYLVAWHGYGTGLHAPGEKGNVAAVYTVGHNLLKAHSKVWHNYNRNFRPHQKGWLSITLGSHWIEPNRAESIVDILKCQQSMVSVLGWFANPIHGDGDYPEVMTKKLLSVLPAFSEAEKNEVRGTADFFAFSFGPNNFKPLNTMAKMGQNVSLNLRQVLNWIKLEYGNPRILIAENGWFTDSYVQTEDTTAIYMMKNFLNQVLQAIRLDGVRVFGYTAWSLLDGFEWQDAYNTRRGLFYVDFNSEQRERRPKSSAHYYKQVIGENGFTLREATPDLQGQFPCDFSWGVTESVLKPESVASSPQFSDPHLYVWNATGNRMLHRVEGVRLKTRPAQCTDFITIKKQLEMLARMKVTHFRFALDWASVLPTGNLSEVNRQALRYYRCVVTEGLKLNISPMVTLYYPTHAHLGLPAPLLHSGGWLDPSTAKAFRDYAGLCFRELGDLVKLWITINEPNRLSDVYNRTSNDTYQAAHNLLIAHAIVWHLYDRQYRPSQRGALSLSLHSDWAEPANPYVASHWQAAERFLQFEIAWFAEPLFKTGDYPVAMREYIASKTRRGLSSSVLPRFSDAERRLVKGAADFYALNHFTTRFVMHEQQNGSRYDSDRDVQFLQDITRLASPSRLAVMPWGEGKLLRWMRNNYGDLDVYITANGIDDQALQNDQLRQYYLEKYVQEALKAYLIDKIKIKGYYAFKLTEEKSKPRFGFFTSDFKAKSSIQFYNKLITSNGFPSENGGPRCNQTQGNPECTVCLLLL

SEQ ID NO: 149 - protein, 950 aa, synthetic construct
  REGION 1..950: note = source = /note="Description of Artificial Sequence: Syntheticpolypeptide"
DYKDDDDKLEFSGDGRAVWSKNPNFTPVNESQLFLYDTFPKNFFWGVGTGALQVEGSWKKDGKGPSIWDHFVHTHLKNVSSTNGSSDSYIFLEKDLSALDFIGVSFYQFSISWPRLFPDGIVTVANAKGLQYYNTLLDSLVLRNIEPIVTLYHWDLPLALQEKYGGWKNDTIIDIFNDYATYCFQTFGDRVKYWITIHNPYLVAWHGYGTGMHAPGEKGNLAAVYTVGHNLIKAHSKVWHNYNTHFRPHQKGWLSITLGSHWIEPNRSENTMDILKCQQSMVSVLGWFASPIHGDGDYPEGMKKKLLSILPLFSEAEKNEVRGTADFFAFSFGPNNFKPLNTMAKMGQNVSLNLREALNWIKLEYNNPRILIAENGWFTDSHVKTEDTTAIYMMKNFLSQVLQAIRLDEIRVFGYTAWSLLDGFEWQDAYTIRRGLFYVDFNSKQKERKPKSSAHYYKQIIRENGFSLKEATPDVQGQFPCDFSWGVTESVLKPESVASSPQFSDPYLYVWNATGNRLLHRVEGVRLKTRPAQCTDFVNIKKQLEMLARMKVTHYRFALDWASVLPTGNLSAVNRQALRYYRCVVSEGLKLGISAMVTLYYPTHAHLGLPEPLLHAGGWLNPSTVEAFQAYAGLCFQELGDLVKLWITINEPNRLSDIYNRSGNDTYGAAHNLLVAHALAWRLYDRQFRPSQRGAVSLSLHADWAEPANPYADSHWRAAERFLQFEIAWFAEPLFKTGDYPAAMREYIASKHRRGLSSSALPRLTEAERRLLKGTVDFCALNHFTTRFVMHEQLAGSRYDSDRDIQFLQDITRLSSPTRLAVIPWGVRKLLRWVRRNYGDMDIYITASGIDDQALEDDRLRKYYLEKYLQEVLKAYLIDKVRIKGYYAFKLAEEKSKPRFGFFTSDFKAKSSIQFYNKMISSSGFPSENSSSRCSQTQKNTECTVCLFLA

SEQ ID NO: 150 - protein, 950 aa, synthetic construct
  REGION 1..950: note = source = /note="Description of Artificial Sequence: Syntheticpolypeptide"
DYKDDDDKLEFSGDGRAVWSKNPNFTPVNESQLFLYDTFPKNFFWGVGTGALQVEGSWKKDGKGPSIWDHFVHTHLKNVSSTNGSSDSYIFLEKDLSALDFIGVSFYQFSISWPRLFPDGIVTVANAKGLQYYNALLDSLVLRNIEPIVTLYHWDLPLALQEKYGGWKNDTIIDIFNDYATYCFQTFGDRVKYWITIHNPYLVAWHGYGTGMHAPGEKGNLAAVYTVGHNLIKAHSKVWHNYNTHFRPHQKGWLSITLGSHWIEPNRSENTMDILKCQQSMVSVLGWFANPIHGDGDYPEGMKKKLLSILPLFSEAEKNEVRGTADFFAFSFGPNNFKPLNTMAKMGQNVSLNLREALNWIKLEYNNPQILIAENGWFTDSHVKTEDTTAIYMMKNFLSQVLQAIRLDEIRVFGYTAWSLLDGFEWQDAYTIRRGLFYVDFNSKQKERKPKSSAHYYKQIIRENGFSLKEATPDVQGQFPCDFSWGVTESVLKPESVASSPQFSDPYLYVWNATGNRLLHRVEGVRLKTRPAQCTDFVNIKKQLEMLARMKVTHYRFALDWASVLPTGNLSAVNRQALRYYRCVVSEGLKLGISAMVTLYYPTHAHLGLPEPLLHAGGWLNPSTVEAFQAYAGLCFQELGDLVKLWITINEPNRLSDIYNRSGNDTYGAAHNLLVAHALAWRLYDRQFRPSQRGAVSLSLHADWAEPANPYADSHWRAAERFLQFEIAWFAEPLFKTGDYPAAMREYIASKHRRGLSSSALPRLTEAERRLLKGTVDFCALNHFTTRFVMHEQLAGSRYDSDRDIQFLQDITRLSSPTRLAVIPWGVRKLLRWVRRNYGDMDIYITASGIDDQALEDDRLRKYYLEKYLQEVLKAYLIDKVRIKGYYAFKLAEEKSKPRFGFFTSDFKAKSSIQFYNKMISSSGFPSENSSSRCSQTQKNTECTVCLFLV

SEQ ID NO: 151 - protein, 989 aa, synthetic construct
  REGION 1..989: note = source = /note="Description of Artificial Sequence: Syntheticpolypeptide"
EPGDGAQTWARFSRPPAPEAAGLFQGTFPDGFLWAVGSAAYQTEGGWQQHGKGASIWDTFTHHPLAPPGDSRNASLPLGAPSPLQPATGDVASDSYNNVFRDTEALRELGVTHYRFSISWARVLPNGSAGVPNREGLRYYRRLLERLRELGVQPVVTLYHWDLPQRLQDAYGGWANRALADHFRDYAELCFRHFGGQVKYWITIDNPYVVAWHGYATGRLAPGIRGSPRLGYLVAHNLLLAHAKVWHLYNTSFRPTQGGQVSIALSSHWINPRRMTDHSIKECQKSLDFVLGWFAKPVFIDGDYPESMKNNLSSILPDFTESEKKFIKGTADFFALCFGPTLSFQLLDPHMKFRQLESPNLRQLLSWIDLEFNHPQIFIVENGWFVSGTTKRDDAKYMYYLKKFIMETLKAIKLDGVDVIGYTAWSLMDGFEWHRGYSIRRGLFYVDFLSQDKMLLPKSSALFYQKLIEKNGFPPLPENQPLEGTFPCDFAWGVVDNYIQVDTTLSQFTDLNVYLWDVHHSKRLIKVDGVVTKKRKSYCVDFAAIQPQIALLQEMHVTHFRFSLDWALILPLGNQSQVNHTILQYYRCMASELVRVNITPVVALWQPMAPNQGLPRLLARQGAWENPYTALAFAEYARLCFQELGHHVKLWITMNEPYTRNMTYSAGHNLLKAHALAWHVYNEKFRHAQNGKISIALQADWIEPACPFSQKDKEVAERVLEFDIGWLAEPIFGSGDYPWVMRDWLNQRNNFLLPYFTEDEKKLIQGTFDFLALSHYTTILVDSEKEDPIKYNDYLEVQEMTDITWLNSPSQVAVVPWGLRKVLNWLKFKYGDLPMYIISNGIDDGLHAEDDQLRVYYMQNYINEALKAHILDGINLCGYFAYSFNDRTAPRFGLYRYAADQFEPKASMKHYRKIIDSNGFPGPETLERFCPEEFTVCTECSFFHTRKSLLAFIAFLFFASIISLSLIFYYSKKGRRSYKLEDYKDDDDK

SEQ ID NO: 152 - protein, 5 aa, synthetic construct
  REGION 1..5: note = source = /note="Description of Artificial Sequence: Syntheticpeptide"
STYIS

SEQ ID NO: 153 - protein, 17 aa, synthetic construct
  REGION 1..17: note = source = /note="Description of Artificial Sequence: Syntheticpeptide"
EIDPYDGATDYADSVKG

SEQ ID NO: 154 - protein, 14 aa, synthetic construct
  REGION 1..14: note = source = /note="Description of Artificial Sequence: Syntheticpeptide"
EHFDAWVHYYVMDY

SEQ ID NO: 155 - protein, 455 aa, Homo sapiens
FPCDFSWGVTESVLKPESVASSPQFSDPHLYVWNATGNRLLHRVEGVRLKTRPAQCTDFVNIKKQLEMLARMKVTHYRFALDWASVLPTGNLSAVNRQALRYYRCVVSEGLKLGISAMVTLYYPTHAHLGLPEPLLHADGWLNPSTAEAFQAYAGLCFQELGDLVKLWITINEPNRLSDIYNRSGNDTYGAAHNLLVAHALAWRLYDRQFRPSQRGAVSLSLHADWAEPANPYADSHWRAAERFLQFEIAWFAEPLFKTGDYPAAMREYIASKHRRGLSSSALPRLTEAERRLLKGTVDFCALNHFTTRFVMHEQLAGSRYDSDRDIQFLQDITRLSSPTRLAVIPWGVRKLLRWVRRNYGDMDIYITASGIDDQALEDDRLRKYYLGKYLQEVLKAYLIDKVRIKGYYAFKLAEEKSKPRFGFFTSDFKAKSSIQFYNKVISSRGFPFENSSSR

SEQ ID NO: 156 - DNA, 36 bp, Mus sp.
  source 1..36: mol_type = unassigned DNA
gttaccggcttctccggagacgggaaagcaatatgg

SEQ ID NO: 157 - protein, 52 aa, Homo sapiens
MKPGCAAGSPGNEWIFFSTDEITTRYRNTMSNGGLQRSVILSALILLRAVTG

SEQ ID NO: 158 - protein, 938 aa, Mus sp.
FSGDGKAIWDKKQYVSPVNPSQLFLYDTFPKNFSWGVGTGAFQVEGSWKTDGRGPSIWDRYVYSHLRGVNGTDRSTDSYIFLEKDLLALDFLGVSFYQFSISWPRLFPNGTVAAVNAQGLRYYRALLDSLVLRNIEPIVTLYHWDLPLTLQEEYGGWKNATMIDLFNDYATYCFQTFGDRVKYWITIHNPYLVAWHGFGTGMHAPGEKGNLTAVYTVGHNLIKAHSKVWHNYDKNFRPHQKGWLSITLGSHWIEPNRTDNMEDVINCQHSMSSVLGWFANPIHGDGDYPEFMKTGAMIPEFSEAEKEEVRGTADFFAFSFGPNNFRPSNTVVKMGQNVSLNLRQVLNWIKLEYDDPQILISENGWFTDSYIKTEDTTAIYMMKNFLNQVLQAIKFDEIRVFGYTAWTLLDGFEWQDAYTTRRGLFYVDFNSEQKERKPKSSAHYYKQIIQDNGFPLKESTPDMKGRFPCDFSWGVTESVLKPEFTVSSPQFTDPHLYVWNVTGNRLLYRVEGVRLKTRPSQCTDYVSIKKRVEMLAKMKVTHYQFALDWTSILPTGNLSKVNRQVLRYYRCVVSEGLKLGVFPMVTLYHPTHSHLGLPLPLLSSGGWLNMNTAKAFQDYAELCFRELGDLVKLWITINEPNRLSDMYNRTSNDTYRAAHNLMIAHAQVWHLYDRQYRPVQHGAVSLSLHCDWAEPANPFVDSHWKAAERFLQFEIAWFADPLFKTGDYPSVMKEYIASKNQRGLSSSVLPRFTAKESRLVKGTVDFYALNHFTTRFVIHKQLNTNRSVADRDVQFLQDITRLSSPSRLAVTPWGVRKLLAWIRRNYRDRDIYITANGIDDLALEDDQIRKYYLEKYVQEALKAYLIDKVKIKGYYAFKLTEEKSKPRFGFFTSDFRAKSSVQFYSKLISSSGLPAENRSPACGQPAEDTDCTICSFLV

SEQ ID NO: 159 - protein, 53 aa, Homo sapiens
MEKKLHAVPAAKTVKFKCPSSGTPNPTLRWLKNGKEFKPDHRIGGYKVRYATW

SEQ ID NO: 160 - protein, 34 aa, Homo sapiens; identical to SEQ ID NO: 142

SEQ ID NO: 161 - protein, 34 aa, Macaca fascicularis; identical to SEQ ID NO: 142

SEQ ID NO: 162 - protein, 34 aa, Rattus sp.
SSPSRLAVTPWGMRKLLGWIRRNYRDMDIYVTAN

SEQ ID NO: 163 - protein, 34 aa, Mus sp.
SSPSRLAVTPWGVRKLLAWIRRNYRDRDIYITAN

SEQ ID NO: 164 - protein, 34 aa, unidentified
  REGION 1..34: note = source = /note="Description of Unknown: Rabbit polypeptide"
ASPSRLAVMPWGEGKLLRWMRNNYGDLDVYITAN

SEQ ID NO: 165 - protein, 17 aa, Mus sp.
FSGDGKAIWDKKQYVSP

SEQ ID NO: 166 - protein, 14 aa, synthetic construct
  REGION 1..14: note = source = /note="Description of Artificial Sequence: Syntheticpeptide"
FSETGKQYGIKNST